European Patent Specification EP 3 658 171 B1, published August 30, 2023. Title: Multi-epitope fusion protein of an HCV antigen and uses thereof. Applicant: Roche Diagnostics GmbH F. Hoffmann-La Roche AG Roche Diagnostics Operations, Inc. The sequence listing filed with the application follows.

SEQUENCE LISTING (6 sequences)

SEQ ID NO: 1 - protein, 191 aa, Hepatitis C virus
MSTNPKPQKKNKRNTNRRPQDVKFPGGGQIVGGVYLLPRRGPRLGVRATRKTSERSQPRGRRQPIPKARRPEGRTWAQPGYPWPLYGNEGCGWAGWLLSPRGSRPSWGPTDPRRRSRNLGKVIDTLTCGFADLMGYIPLVGAPLGGAARALAHGVRVLEDGVNYATGNLPGCSFSIFLLALLSCLTVPASA

SEQ ID NO: 2 - protein, 192 aa, Hepatitis C virus
YQVRNSTGLYHVTNDCPNSSIVYEAADAILHTPGCVPCVREGNASRCWVAMTPTVATRDGKLPATQLRRHIDLLVGSATLCSALYVGDLCGSVFLVGQLFTFSPRRHWTTQGCNCSIYPGHITGHRMAWDMMMNWSPTTALVMAQLLRIPQAILDMIAGAHWGVLAGIAYFSMVGNWAKVLVVLLLFAGVDA

SEQ ID NO: 3 - protein, 363 aa, Hepatitis C virus
ETHVTGGSAGHTVSGFVSLLAPGAKQNVQLINTNGSWHLNSTALNCNDSLNTGWLAGLFYHHKFNSSGCPERLASCRPLTDFDQGWGPISYANGSGPDQRPYCWHYPPKPCGIVPAKSVCGPVYCFTPSPVVVGTTDRSGAPTYSWGENDTDVFVLNNTRPPLGNWFGCTWMNSTGFTKVCGAPPCVIGGAGNNTLHCPTDCFRKHPDATYSRCGSGPWITPRCLVDYPYRLWHYPCTINYTIFKIRMYVGGVEHRLEAACNWTRGERCDLEDRDRSELSPLLLTTTQWQVLPCSFTTLPALSTGLIHLHQNIVDVQYLYGVGSSIASWAIKWEYVVLLFLLLADARVCSCLWMMLLISQAEA

SEQ ID NO: 4 - protein, 432 aa, Artificial
  HCV core 3-epitopes calibrator
MRGSGRRQPIPKARRPEGRTGGGSGGGMKVAKDLVVSLAYQVRTEDGVLVDESPVSAPLDYLHGHGSLISGLETALEGHEVGDKFDVAVGANDAYGQYDENLVQRVPKDVFMGVDELQVGMRFLAETDQGPVPVEITAVEDDHVVVDGNHMLAGQNLKFNVEVVAIREATEEELAHGHVHGAHDHHHDHDHDGGGSGGGLLSPRGSRPSWGPTDPRRRSRGGGSGGGMKVAKDLVVSLAYQVRTEDGVLVDESPVSAPLDYLHGHGSLISGLETALEGHEVGDKFDVAVGANDAYGQYDENLVQRVPKDVFMGVDELQVGMRFLAETDQGPVPVEITAVEDDHVVVDGNHMLAGQNLKFNVEVVAIREATEEELAHGHVHGAHDHHHDHDHDGGGSGGGAHGVRVLEDGVNYATGNLPGGGGSGGGHHHHHH

SEQ ID NO: 5 - protein, 473 aa, Artificial Sequence
  HCVcore-3-epitopes calibrator (HCVcore-3Epi-EcS-FP, XY(Z, extralong, C/A))
MRGSGRRQPIPKARRPEGRTGGGSGGGMKVAKDLVVSLAYQVRTEDGVLVDESPVSAPLDYLHGHGSLISGLETALEGHEVGDKFDVAVGANDAYGQYDENLVQRVPKDVFMGVDELQVGMRFLAETDQGPVPVEITAVEDDHVVVDGNHMLAGQNLKFNVEVVAIREATEEELAHGHVHGAHDHHHDHDHDGGGSGGGLLSPRGSRPSWGPTDPRRRSRGGGSGGGMKVAKDLVVSLAYQVRTEDGVLVDESPVSAPLDYLHGHGSLISGLETALEGHEVGDKFDVAVGANDAYGQYDENLVQRVPKDVFMGVDELQVGMRFLAETDQGPVPVEITAVEDDHVVVDGNHMLAGQNLKFNVEVVAIREATEEELAHGHVHGAHDHHHDHDHDGGGSGGGDPRRRSRNLGKVIDTLTAGFADLMGYIPLVGAPLGGAARALAHGVRVLEDGVNYATGNLPGGGGSGGGHHHHHH

SEQ ID NO: 6 - protein, 513 aa, Artificial Sequence
  HCVcore-3-epitopes calibrator (HCVcore-3Epi-EcS-FP, XY(Z)4)
MRGSGRRQPIPKARRPEGRTGGGSGGGMKVAKDLVVSLAYQVRTEDGVLVDESPVSAPLDYLHGHGSLISGLETALEGHEVGDKFDVAVGANDAYGQYDENLVQRVPKDVFMGVDELQVGMRFLAETDQGPVPVEITAVEDDHVVVDGNHMLAGQNLKFNVEVVAIREATEEELAHGHVHGAHDHHHDHDHDGGGSGGGLLSPRGSRPSWGPTDPRRRSRGGGSGGGMKVAKDLVVSLAYQVRTEDGVLVDESPVSAPLDYLHGHGSLISGLETALEGHEVGDKFDVAVGANDAYGQYDENLVQRVPKDVFMGVDELQVGMRFLAETDQGPVPVEITAVEDDHVVVDGNHMLAGQNLKFNVEVVAIREATEEELAHGHVHGAHDHHHDHDHDGGGSGGGAHGVRVLEDGVNYATGNLPGGGGSGGGAHGVRVLEDGVNYATGNLPGGGGSGGGAHGVRVLEDGVNYATGNLPGGGGSGGGAHGVRVLEDGVNYATGNLPGGGGSGGGHHHHHH